European Patent Application EP 4 643 878 A2, published November 5, 2025. Title: PHARMACEUTICAL FORMULATION COMPRISING THERAPEUTIC ANTIBODY AND USE THEREOF. Applicant: Suzhou Transcenta therapeutics Co.,Ltd. Application WO. The sequence listing filed with the application follows.

SEQUENCE LISTING (43 sequences)

SEQ ID NO: 1 - protein, 5 aa, synthetic construct
  REGION 1..5: note = Synthetic
DYYIN

SEQ ID NO: 2 - protein, 17 aa, synthetic construct
  REGION 1..17: note = Synthetic
  SITE 7: note = misc_feature - Xaa can be Glu, Asp or Gly.
  SITE 9: note = misc_feature - Xaa can be Ala or Pro.
  REGION 11..14: note = misc_feature - Xaa at position 11 can be His or Tyr, Xaa at position 12 can be Ser or Asn, Xaa at position 13 can be Glu or Gln, and Xaa at position 14 can be Lys or Asn.
  REGION 16..17: note = misc_feature - Xaa at position 16 can be Lys or Gln, and Xaa at position 17 can be Ala or Gly.
WIFPGSXSXYXXXXFXX

SEQ ID NO: 3 - protein, 9 aa, synthetic construct
  REGION 1..9: note = Synthetic
  SITE 8: note = misc_feature - Xaa can be Ala or Pro.
GDRSGPFXY

SEQ ID NO: 4 - protein, 16 aa, synthetic construct
  REGION 1..16: note = Synthetic
KSSQSLLYSNGKTYLN

SEQ ID NO: 5 - protein, 7 aa, synthetic construct
  REGION 1..7: note = Synthetic
LVSKLDS

SEQ ID NO: 6 - protein, 9 aa, synthetic construct
  REGION 1..9: note = Synthetic
  SITE 3: note = misc_feature - Xaa can be Val or Gly.
VQXTHFPFT

SEQ ID NO: 7 - protein, 17 aa, synthetic construct
  REGION 1..17: note = Synthetic
WIFPGSESAYHSEKFKA

SEQ ID NO: 8 - protein, 17 aa, synthetic construct
  REGION 1..17: note = Synthetic
WIFPGSESAYHSQKFQG

SEQ ID NO: 9 - protein, 17 aa, synthetic construct
  REGION 1..17: note = Synthetic
WIFPGSDSAYYNEKFKG

SEQ ID NO: 10 - protein, 17 aa, synthetic construct
  REGION 1..17: note = Synthetic
WIFPGSGSPYYNENFKG

SEQ ID NO: 11 - protein, 9 aa, synthetic construct
  REGION 1..9: note = Synthetic
GDRSGPFAY

SEQ ID NO: 12 - protein, 9 aa, synthetic construct
  REGION 1..9: note = Synthetic
GDRSGPFPY

SEQ ID NO: 13 - protein, 9 aa, synthetic construct
  REGION 1..9: note = Synthetic
VQVTHFPFT

SEQ ID NO: 14 - protein, 9 aa, synthetic construct
  REGION 1..9: note = Synthetic
VQGTHFPFT

SEQ ID NO: 15 - protein, 118 aa, synthetic construct
  REGION 1..118: note = Synthetic
QVQLQQSGPELEKPGTSVKISCEASGYTFTDYYINWVQQRPGQGLEWIGWIFPGSESAYHSEKFKAKATLTVDTSSTTAYMLLTSLTSEDSAVYFCTRGDRSGPFAYWGQGTLVTVSA

SEQ ID NO: 16 - protein, 112 aa, synthetic construct
  REGION 1..112: note = Synthetic
DVVMTQTPLTLSVTIGQPASISCKSSQSLLYSNGKTYLNWLLQRPGQSPKRLIYLVSKLDSGVPDRFTGSGSGADFTLKISRVEAEDLGVYYCVQVTHFPFTFGTGTKLEIK

SEQ ID NO: 17 - protein, 118 aa, synthetic construct
  REGION 1..118: note = Synthetic
QVQLQQSGPELVKPGASVKISCKASGYTFTDYYINWVKQRPGQGLEWVGWIFPGSDSAYYNEKFKGKATLTVDTSSSTAYMLLSSLTSEDSAVYFCARGDRSGPFPYWGQGTLVTVSA

SEQ ID NO: 18 - protein, 118 aa, synthetic construct
  REGION 1..118: note = Synthetic
QVQLQQSGPDLVKPGTSVKISCTASGYTFTDYYINWVKQRPGQGLEWIGWIFPGSGSPYYNENFKGRAMFTVDYSSSSAYMLLSSLTSEDSAVYFCTRGDRSGPFAYWGQGTLVTVSA

SEQ ID NO: 19 - protein, 112 aa, synthetic construct
  REGION 1..112: note = Synthetic
DVVMTQTPLTLSVTIGQPASISCKSSQSLLYSNGKTYLNWLLQRPGQSPKRLIYLVSKLDSGVPDRFTGSGSGADFTLKISRVEAEDLGVYYCVQGTHFPFTFGTGTKLEIK

SEQ ID NO: 20 - protein, 118 aa, synthetic construct
  REGION 1..118: note = Synthetic
QVQLVQSGAEVKKPGASVKVSCKASGYTFTDYYINWVRQAPGQGLEWMGWIFPGSESAYHSEKFKARVTMTVDTSISTAYMELSRLRSDDTAVYYCTRGDRSGPFAYWGQGTLVTVSS

SEQ ID NO: 21 - skipped

SEQ ID NO: 22 - protein, 118 aa, synthetic construct
  REGION 1..118: note = Synthetic
QVQLVQSGAEVKKPGASVKVSCKASGYTFTDYYINWVRQAPGQGLEWMGWIFPGSESAYHSEKFKARATLTVDTSISTAYMELSRLRSDDTAVYYCTRGDRSGPFAYWGQGTLVTVSS

SEQ ID NO: 23 - skipped

SEQ ID NO: 24 - protein, 118 aa, synthetic construct
  REGION 1..118: note = Synthetic
QVQLVQSGAEVKKPGASVKVSCKASGYTFTDYYINWVRQAPGQGLEWMGWIFPGSESAYHSQKFQGRVTMTVDTSISTAYMELSRLRSDDTAVYYCTRGDRSGPFAYWGQGTLVTVSS

SEQ ID NO: 25 - skipped

SEQ ID NO: 26 - protein, 118 aa, synthetic construct
  REGION 1..118: note = Synthetic
QVQLVQSGAEVKKPGASVKVSCKASGYTFTDYYINWVRQAPGQGLEWMGWIFPGSESAYHSQKFQGRATLTVDTSISTAYMELSRLRSDDTAVYYCTRGDRSGPFAYWGQGTLVTVSS

SEQ ID NO: 27 - skipped

SEQ ID NO: 28 - protein, 112 aa, synthetic construct
  REGION 1..112: note = Synthetic
DVVMTQSPLSLPVTLGQPASISCKSSQSLLYSNGKTYLNWLQQRPGQSPRRLIYLVSKLDSGVPDRFSGSGSGTDFTLKISRVEAEDVGVYYCVQVTHFPFTFGQGTKLEIK

SEQ ID NO: 29 - protein, 219 aa, synthetic construct
  REGION 1..219: note = Synthetic
DVVMTQSPLSLPVTLGQPASISCKSSQSLLYSNGKTYLNWLQQRPGQSPRRLIYLVSKLDSGVPDRFSGSGSGTDFTLKISRVEAEDVGVYYCVQVTHFPFTFGQGTKLEIKRTVAAPSVFIFPPSDEQLKSGTASVVCLLNNFYPREAKVQWKVDNALQSGNSQESVTEQDSKDSTYSLSSTLTLSKADYEKHKVYACEVTHQGLSSPVTKSFNRGEC

SEQ ID NO: 30 - protein, 112 aa, synthetic construct
  REGION 1..112: note = Synthetic
DVVMTQSPLSLPVTLGQPASISCKSSQSLLYSNGKTYLNWLQQRPGQSPRRLIYLVSKLDSGVPDRFSGSGSGADFTLKISRVEAEDVGVYYCVQVTHFPFTFGQGTKLEIK

SEQ ID NO: 31 - skipped

SEQ ID NO: 32 - protein, 445 aa, synthetic construct
  REGION 1..445: note = Synthetic
QVTLKESGPVLVKPTETLTLTCTVSGFSLSRGKMGVSWIRQPPGKALEWLAHIFSSDEKSYRTSLKSRLTISKDTSKNQVVLTMTNMDPVDTATYYCARIRRGGIDYWGQGTLVTVSSASTKGPSVFPLAPCSRSTSESTAALGCLVKDYFPEPVTVSWNSGALTSGVHTFPAVLQSSGLYSLSSVVTVPSSSLGTKTYTCNVDHKPSNTKVDKRVESKYGPPCPPCPAPEFLGGPSVFLFPPKPKDTLMISRTPEVTCVVVDVSQEDPEVQFNWYVDGVEVHNAKTKPREEQFNSTYRVVSVLTVLHQDWLNGKEYKCKVSNKGLPSSIEKTISKAKGQPREPQVYTLPPSQEEMTKNQVSLTCLVKGFYPSDIAVEWESNGQPENNYKTTPPVLDSDGSFFLYSRLTVDKSRWQEGNVFSCSVMHEALHNHYTQKSLSLSLGK

SEQ ID NO: 33 - protein, 213 aa, synthetic construct
  REGION 1..213: note = Synthetic
QPVLTQPPSLSVSPGQTASITCSGEKLGDKYAYWYQQKPGQSPVLVMYQDKQRPSGIPERFSGSNSGNTATLTISGTQAMDEADYYCQAWDSSTAVFGGGTKLTVLRTVAAPSVFIFPPSDEQLKSGTASVVCLLNNFYPREAKVQWKVDNALQSGNSQESVTEQDSKDSTYSLSSTLTLSKADYEKHKVYACEVTHQGLSSPVTKSFNRGEC

SEQ ID NO: 34 - protein, 107 aa, Homo sapiens [sequence omitted]

SEQ ID NO: 35 - protein, 327 aa, synthetic construct
  REGION 1..327: note = Synthetic
ASTKGPSVFPLAPCSRSTSESTAALGCLVKDYFPEPVTVSWNSGALTSGVHTFPAVLQSSGLYSLSSVVTVPSSSLGTKTYTCNVDHKPSNTKVDKRVESKYGPPCPPCPAPEFLGGPSVFLFPPKPKDTLYITREPEVTCVVVDVSQEDPEVQFNWYVDGVEVHNAKTKPREEQFNSTYRVVSVLTVLHQDWLNGKEYKCKVSNKGLPSSIEKTISKAKGQPREPQVYTLPPSQEEMTKNQVSLTCLVKGFYPSDIAVEWESNGQPENNYKTTPPVLDSDGSFFLYSRLTVDKSRWQEGNVFSCSVMHEALHNHYTQKSLSLSLGK

SEQ ID NO: 36 - protein, 445 aa, synthetic construct
  REGION 1..445: note = Synthetic
QVQLVQSGAEVKKPGASVKVSCKASGYTFTDYYINWVRQAPGQGLEWMGWIFPGSESAYHSEKFKARVTMTVDTSISTAYMELSRLRSDDTAVYYCTRGDRSGPFAYWGQGTLVTVSSASTKGPSVFPLAPCSRSTSESTAALGCLVKDYFPEPVTVSWNSGALTSGVHTFPAVLQSSGLYSLSSVVTVPSSSLGTKTYTCNVDHKPSNTKVDKRVESKYGPPCPPCPAPEFLGGPSVFLFPPKPKDTLYITREPEVTCVVVDVSQEDPEVQFNWYVDGVEVHNAKTKPREEQFNSTYRVVSVLTVLHQDWLNGKEYKCKVSNKGLPSSIEKTISKAKGQPREPQVYTLPPSQEEMTKNQVSLTCLVKGFYPSDIAVEWESNGQPENNYKTTPPVLDSDGSFFLYSRLTVDKSRWQEGNVFSCSVMHEALHNHYTQKSLSLSLGK

SEQ ID NO: 37 - protein, 98 aa, Homo sapiens
QVQLVQSGAEVKKPGASVKVSCKASGYTFTGYYMHWVRQAPGQGLEWMGWINPNSGGTNYAQKFQGRVTMTRDTSISTAYMELSRLRSDDTAVYYCAR

SEQ ID NO: 38 - protein, 100 aa, Homo sapiens
DVVMTQSPLSLPVTLGQPASISCRSSQSLVYSDGNTYLNWFQQRPGQSPRRLIYKVSNRDSGVPDRFSGSGSGTDFTLKISRVEAEDVGVYYCMQGTHWP

SEQ ID NO: 39 - protein, 686 aa, Homo sapiens
MRLLTLLGLLCGSVATPLGPKWPEPVFGRLASPGFPGEYANDQERRWTLTAPPGYRLRLYFTHFDLELSHLCEYDFVKLSSGAKVLATLCGQESTDTERAPGKDTFYSLGSSLDITFRSDYSNEKPFTGFEAFYAAEDIDECQVAPGEAPTCDHHCHNHLGGFYCSCRAGYVLHRNKRTCSALCSGQVFTQRSGELSSPEYPRPYPKLSSCTYSISLEEGFSVILDFVESFDVETHPETLCPYDFLKIQTDREEHGPFCGKTLPHRIETKSNTVTITFVTDESGDHTGWKIHYTSTAQPCPYPMAPPNGHVSPVQAKYILKDSFSIFCETGYELLQGHLPLKSFTAVCQKDGSWDRPMPACSIVDCGPPDDLPSGRVEYITGPGVTTYKAVIQYSCEETFYTMKVNDGKYVCEADGFWTSSKGEKSLPVCEPVCGLSARTTGGRIYGGQKAKPGDFPWQVLILGGTTAAGALLYDNWVLTAAHAVYEQKHDASALDIRMGTLKRLSPHYTQAWSEAVFIHEGYTHDAGFDNDIALIKLNNKVVINSNITPICLPRKEAESFMRTDDIGTASGWGLTQRGFLARNLMYVDIPIVDHQKCTAAYEKPPYPRGSVTANMLCAGLESGGKDSCRGDSGGALVFLDSETERWFVGGIVSWGSMNCGEAGQYGVYTKVINYIPWIENIISDF

SEQ ID NO: 40 - protein, 685 aa, Mus musculus
MRLLIFLGLLWSLVATLLGSKWPEPVFGRLVSPGFPEKYADHQDRSWTLTAPPGYRLRLYFTHFDLELSYRCEYDFVKLSSGTKVLATLCGQESTDTEQAPGNDTFYSLGPSLKVTFHSDYSNEKPFTGFEAFYAAEDVDECRVSLGDSVPCDHYCHNYLGGYYCSCRAGYVLHQNKHTCSALCSGQVFTGRSGYLSSPEYPQPYPKLSSCTYSIRLEDGFSVILDFVESFDVETHPEAQCPYDSLKIQTDKGEHGPFCGKTLPPRIETDSHKVTITFATDESGNHTGWKIHYTSTARPCPDPTAPPNGSISPVQAIYVLKDRFSVFCKTGFELLQGSVPLKSFTAVCQKDGSWDRPMPECSIIDCGPPDDLPNGHVDYITGPEVTTYKAVIQYSCEETFYTMSSNGKYVCEADGFWTSSKGEKLPPVCEPVCGLSTHTIGGRIVGGQPAKPGDFPWQVLLLGQTTAAAGALIHDNWVLTAAHAVYEKRMAASSLNIRMGILKRLSPHYTQAWPEEIFIHEGYTHGAGFDNDIALIKLKNKVTINGSIMPVCLPRKEAASLMRTDFTGTVAGWGLTQKGLLARNLMFVDIPIADHQKCTAVYEKLYPGVRVSANMLCAGLETGGKDSCRGDSGGALVFLDNETQRWFVGGIVSWGSINCGAADQYGVYTKVINYIPWIENIISNF

SEQ ID NO: 41 - protein, 20 aa, Homo sapiens
MYRMQLLSCIALSLALVTNS

SEQ ID NO: 42 - protein, 695 aa, synthetic construct
  REGION 1..695: note = Synthetic
MYRMQLLSCIALSLALVTNSSKWPEPVFGRLVSPGFPEKYADHQDRSWTLTAPPGYRLRLYFTHFDLELSYRCEYDFVKLSSGTKVLATLCGQESTDTEQAPGNDTFYSLGPSLKVTFHSDYSNEKPFTGFEAFYAAEDVDECRVSLGDSVPCDHYCHNYLGGYYCSCRAGYVLHQNKHTCSALCSGQVFTGRSGYLSSPEYPQPYPKLSSCTYSIRLEDGFSVILDFVESFDVETHPEAQCPYDSLKIQTDKGEHGPFCGKTLPPRIETDSHKVTITFATDESGNHTGWKIHYTSTAQPCPYPMAPPNGHVSPVQAKYILKDSFSIFCETGYELLQGHLPLKSFTAVCQKDGSWDRPMPACSIVDCGPPDDLPSGRVEYITGPGVTTYKAVIQYSCEETFYTMKVNDGKYVCEADGFWTSSKGEKSLPVCEPVCGLSARTTGGRIYGGQKAKPGDFPWQVLILGGTTAAGALLYDNWVLTAAHAVYEQKHDASALDIRMGTLKRLSPHYTQAWSEAVFIHEGYTHDAGFDNDIALIKLNNKVVINSNITPICLPRKEAESFMRTDDIGTASGWGLTQRGFLARNLMYVDIPIVDHQKCTAAYEKPPYPRGSVTANMLCAGLESGGKDSCRGDSGGALVFLDSETERWFVGGIVSWGSMNCGEAGQYGVYTKVINYIPWIENIISDFDYKDDDDK

SEQ ID NO: 43 - protein, 686 aa, Macaca fascicularis
MRLLTLLGLLCGSVATPLGPKWPEPVFGRLASPGFPGEYANDQERRWTLTAPPGYRLRLYFTHFDLELSHLCEYDFVKLSSGAKVLATLCGHESTDTERAPGNDTFYSLGSSLDITFRSDYSNEKPFTGFEAFYAAEDIDECQVAPGEAPACDHHCHNHLGGFYCSCRVGYILHRNKRTCSALCSGQVFTQRSGELSSPEYPQPYPKLSSCTYSIRLEEGFSVILDFVESFDVETHPETLCPYDFLKIQIDSEEHGPFCGKTLPRRIETKSNTVTITFVTDESGDHTGWKIHYTSTAQPCPYPMAPPNGHLSPVQAKYILKDSFSIFCEPGYELLQGHLPLKSFAAVCQKDGSWDQPMPSCSIVDCGPPDDLPSGRVEYITGPEVTTYKAVIQYSCEETFYTMKVNDGKYVCEADGFWTSSKGERSPPVCEPVCGLSARTTGGRIYGGQKAKPGDFPWQVLILGGSTAAGALLYDNWVLTAAHAIYEQKHDASSLDIRLGALKRLSPHYTQAWAEAVFIHEGYTHDAGFDNDIALIKLNNKVVINSNITPICLPRKEAESFMRTDDIGTASGWGLTQRGLLARNLMYVDIPIVDHQKCTAAYEKPPYSGGSVTANMLCAGLESGGKDSCRGDSGGALVFLDNETQRWFVGGIVSWGSMNCGEAGQYGVYTKVINYIPWIKNIISNF